European Patent Specification EP 3 678 666 B1, published July 9, 2025. Title: SPECIFIC AKT3 ACTIVATORS AND USES THEREOF. Applicant: Augusta University Research Institute, Inc Khleif, Samir N Mkrtichyan, Mikayel. The sequence listing filed with the application follows.

SEQUENCE LISTING (3 sequences)

SEQ ID NO: 1 - DNA, 1708 bp, Homo sapiens
aggggagtcatcatgagcgatgttaccattgtgaaggaaggttgggttcagaagaggggagaatatataaaaaactggaggccaagatacttccttttgaagacagatggctcattcataggatataaagagaaacctcaagatgtggatttaccttatcccctcaacaacttttcagtggcaaaatgccagttaatgaaaacagaacgaccaaagccaaacacatttataatcagatgtctccagtggactactgttatagagagaacatttcatgtagatactccagaggaaagggaagaatggacagaagctatccaggctgtagcagacagactgcagaggcaagaagaggagagaatgaattgtagtccaacttcacaaattgataatataggagaggaagagatggatgcctctacaacccatcataaaagaaagacaatgaatgattttgactatttgaaactactaggtaaaggcacttttgggaaagttattttggttcgagagaaggcaagtggaaaatactatgctatgaagattctgaagaaagaagtcattattgcaaaggatgaagtggcacacactctaactgaaagcagagtattaaagaacactagacatccctttttaacatccttgaaatattccttccagacaaaagaccgtttgtgttttgtgatggaatatgttaatgggggcgagctgtttttccatttgtcgagagagcgggtgttctctgaggaccgcacacgtttctatggtgcagaaattgtctctgccttggactatctacattccggaaagattgtgtaccgtgatctcaagttggagaatctaatgctggacaaagatggccacataaaaattacagattttggactttgcaaagaagggatcacagatgcagccaccatgaagacattctgtggcactccagaatatctggcaccagaggtgttagaagataatgactatggccgagcagtagactggtggggcctaggggttgtcatgtatgaaatgatgtgtgggaggttacctttctacaaccaggaccatgagaaactttttgaattaatattaatggaagacattaaatttcctcgaacactctcttcagatgcaaaatcattgctttcagggctcttgataaaggatccaaataaacgccttggtggaggaccagatgatgcaaaagaaattatgagacacagtttcttctctggagtaaactggcaagatgtatatgataaaaagcttgtacctccttttaaacctcaagtaacatctgagacagatactagatattttgatgaagaatttacagctcagactattacaataacaccacctgaaaaatatgatgaggatggtatggactgcatggacaatgagaggcggccgcatttccctcaattttcctactctgcaagtggacgagaataagtctctttcattctgctacttcactgtcatcttcaatttattactgaaaatgattcctggacatcaccagtcctagctcttacacatagcaggggcaccttccgacatcccagaccagccaagggtcctcacccctcgccacctttcaccctcatgaaaacacacatacacgcaaatacactccagtttttgtttttgcatgaaattgtatctcagtctaaggtctcatgctgttgctgctactgtcttactatta

SEQ ID NO: 2 - protein, 479 aa, Homo sapiens
MSDVTIVKEGWVQKRGEYIKNWRPRYFLLKTDGSFIGYKEKPQDVDLPYPLNNFSVAKCQLMKTERPKPNTFIIRCLQWTTVIERTFHVDTPEEREEWTEAIQAVADRLQRQEEERMNCSPTSQIDNIGEEEMDASTTHHKRKTMNDFDYLKLLGKGTFGKVILVREKASGKYYAMKILKKEVIIAKDEVAHTLTESRVLKNTRHPFLTSLKYSFQTKDRLCFVMEYVNGGELFFHLSRERVFSEDRTRFYGAEIVSALDYLHSGKIVYRDLKLENLMLDKDGHIKITDFGLCKEGITDAATMKTFCGTPEYLAPEVLEDNDYGRAVDWWGLGVVMYEMMCGRLPFYNQDHEKLFELILMEDIKFPRTLSSDAKSLLSGLLIKDPNKRLGGGPDDAKEIMRHSFFSGVNWQDVYDKKLVPPFKPQVTSETDTRYFDEEFTAQTITITPPEKYDEDGMDCMDNERRPHFPQFSYSASGRE

SEQ ID NO: 3 - protein, 478 aa, Homo sapiens
SDVTIVKEGWVQKRGEYIKNWRPRYFLLKTDGSFIGYKEKPQDVDLPYPLNNFSVAKCQLMKTERPKPNTFIIRCLQWTTVIERTFHVDTPEEREEWTEAIQAVADRLQRQEEERMNCSPTSQIDNIGEEEMDASTTHHKRKTMNDFDYLKLLGKGTFGKVILVREKASGKYYAMKILKKEVIIAKDEVAHTLTESRVLKNTRHPFLTSLKYSFQTKDRLCFVMEYVNGGELFFHLSRERVFSEDRTRFYGAEIVSALDYLHSGKIVYRDLKLENLMLDKDGHIKITDFGLCKEGITDAATMKTFCGTPEYLAPEVLEDNDYGRAVDWWGLGVVMYEMMCGRLPFYNQDHEKLFELILMEDIKFPRTLSSDAKSLLSGLLIKDPNKRLGGGPDDAKEIMRHSFFSGVNWQDVYDKKLVPPFKPQVTSETDTRYFDEEFTAQTITITPPEKYDEDGMDCMDNERRPHFPQFSYSASGRE